European Patent Specification EP 3 708 172 B1, published September 10, 2025. Title: PHARMACEUTICAL COMPOSITION FOR PREVENTING OR TREATING ADVERSE DRUG REACTIONS BY STATIN. Applicant: Industry-Academic Cooperation Foundation, Yonsei University. Application EP 18 872 034.6. The sequence listing filed with the application follows.

SEQUENCE LISTING (4 sequences)

SEQ ID NO: 1 - DNA, 20 bp, Artificial Sequence
  HMG-CoA reductase forward primer
caggatgcagcacagaatgt

SEQ ID NO: 2 - DNA, 20 bp, Artificial Sequence
  HMG-CoA reductase reverse primer
ctttgcatgctccttgaaca

SEQ ID NO: 3 - DNA, 20 bp, Artificial Sequence
  GAPDH forward primer
gcacagtcaaggccgagaat

SEQ ID NO: 4 - DNA, 20 bp, Artificial Sequence
  GAPDH reverse primer
gccttctccatggtggtgaa